European Patent Specification EP 3 162 894 B1, published January 10, 2024. Title: Methods for the manufacture of proteolytically processed polypeptides. Applicant: Syntaxin Limited. Application Not yet assigned. The sequence listing filed with the application follows.

SEQUENCE LISTING (27 sequences)

SEQ ID NO: 1 - protein, 333 aa, Clostridium Botulinum
VQGQSVKGVGKTSLDGLVNIDVTYGNGKYYLKDSNKNIYLYDLKNQVDEYDLYNYLSRPNYKQILMSKSELISNYNNNFIANNQVNSVDAYVNTNKTYDYYKNKLNRNSIDNKGMNINGFVHVGRNYGNAFWYGPYDGMFFGDGDGIYFSSLAKSLDVVGHELSHGVTNKESNLKYENESGALNESFSDIMGVAVEGKNFVLGEDCWVAGGVMRDMENPSRGGQPAHMKDYKYKTMNDDNGGVHTNSGIINHAAYLVADGIEKTGAKNSKDIMGKIFYTANCYKWDETTNFAKCRNDVVQVTKELYGENSNYVKIVEKAFDQVGITATPQLPL

SEQ ID NO: 2 - protein, 581 aa, Clostridium Botulinum
MKSKKLLATVLSAVITFSTVSAVYAAPVGKESKVEPKTTTITWEKNEQNTKKAATDITEKKFNNSEEITKFFEKNISKFGVQKGSLKNTKTVKDEKGKTNYHMIYEVEGIPVYYGRIVFTTEKDSSMDSINGRIDTVFENGNWKNKIKLSKEDAIAKAKNDIKDEKATSKKTDLYLYNFEGKPYVVYLVDLITDNGSWTVFVNAEDGSIVNKFNNTPTLIDTKDQKLPNAKKIKDEAKKASNANNVIDVQGQSVKGVGKTSLDGLVNIDVTYGNGKYYLKDSNKNIYLYDLKNQVDEYDLYNYLSRPNYKQILMSKSELISNYNNNFIANNQVNSVDAYVNTNKTYDYYKNKLNRNSIDNKGMNINGFVHVGRNYGNAFWYGPYDGMFFGDGDGIYFSSLAKSLDVVGHELSHGVTNKESNLKYENESGALNESFSDIMGVAVEGKNFVLGEDCWVAGGVMRDMENPSRGGQPAHMKDYKYKTMNDDNGGVHTNSGIINHAAYLVADGIEKTGAKNSKDIMGKIFYTANCYKWDETTNFAKCRNDVVQVTKELYGENSNYVKIVEKAFDQVGITATPQLPL

SEQ ID NO: 3 - protein, 1296 aa, Clostridium Botulinum
MPFVNKQFNYKDPVNGVDIAYIKIPNAGQMQPVKAFKIHNKIWVIPERDTFTNPEEGDLNPPPEAKQVPVSYYDSTYLSTDNEKDNYLKGVTKLFERIYSTDLGRMLLTSIVRGIPFWGGSTIDTELKVIDTNCINVIQPDGSYRSEELNLVIIGPSADIIQFECKSFGHEVLNLTRNGYGSTQYIRFSPDFTFGFEESLEVDTNPLLGAGKFATDPAVTLAHELIHAGHRLYGIAINPNRVFKVNTNAYYEMSGLEVSFEELRTFGGHDAKFIDSLQENEFRLYYYNKFKDIASTLNKAKSIVGTTASLQYMKNVFKEKYLLSEDTSGKFSVDKLKFDKLYKMLTEIYTEDNFVKFFKVLNRKTYLNFDKAVFKINIVPKVNYTIYDGFNLRNTNLAANFNGQNTEINNMNFTKLKNFTGLFEFYKLLCVRGIITSKTKSLDKGYNKALNDLCIKVNNWDLFFSPSEDNFTNDLNKGEEITSDTNIEAAEENISLDLIQQYYLTFNFDNEPENISIENLSSDIIGQLELMPNIERFPNGKKYELDKYTMFHYLRAQEFEHGKSRIALTNSVNEALLNPSRVYTFFSSDYVKKVNKATEAAMFLGWVEQLVYDFTDETSEVSTTDKIADITIIIPYIGPALNIGNMLYKDDFVGALIFSGAVILLEFIPEIAIPVLGTFALVSYIANKVLTVQTIDNALSKRNEKWDEVYKYIVTNWLAKVNTQIDLIRKKMKEALENQAEATKAIINYQYNQYTEEEKNNINFNIDDLSSKLNESINKAMININKFLNQCSVSYLMNSMIPYGVKRLEDFDASLKDALLKYIYDNRGTLIGQVDRLKDKVNNTLSTDIPFQLSKYVDNQRLLSTFTEYIKNIINTSILNLRYESNHLIDLSRYASKINIGSKVNFDPIDKNQIQLFNLESSKIEVILKNAIVYNSMYENFSTSFWIRIPKYFNSISLNNEYTIINCMENNSGWKVSLNYGEIIWTLQDTQEIKQRVVFKYSQMINISDYINRWIFVTITNNRLNNSKIYINGRLIDQKPISNLGNIHASNNIMFKLDGCRDTHRYIWIKYFNLFDKELNEKEIKDLYDNQSNSGILKDFWGDYLQYDKPYYMLNLYDPNKYVDVNNVGIRGYMYLKGPRGSVMTTNIYLNSSLYRGTKFIIKKYASGNKDNIVRNNDRVYINVVVKNKEYRLATNASQAGVEKILSALEIPDVGNLSQVVVMKSKNDQGITNKCKMNLQDNNGNDIGFIGFHQFNNIAKLVASNWYNRQIERSSRTLGCSWEFIPVDDGWGERPL

SEQ ID NO: 4 - protein, 25 aa, Clostridium Botulinum
  Loop BoNT/A1 (1)..(25)
CVRGIITSKTKSLDKGYNKALNDLC

SEQ ID NO: 5 - protein, 25 aa, Clostridium Botulinum
  Loop BoNT/A2/A6 (1)..(25)
CVRGIIPFKTKSLDEGYNKALNDLC

SEQ ID NO: 6 - protein, 25 aa, Clostridium Botulinum
  Loop BoNT/A3 (1)..(25)
CVRGIIPFKTKSLDEGYNKALNDLC

SEQ ID NO: 7 - protein, 25 aa, Clostridium Botulinum
  Loop BoNT/A3 (1)..(25)
CVRGIIPFKTKSLDEGYNKALNYLC

SEQ ID NO: 8 - protein, 25 aa, Clostridium Botulinum
  Loop BoNT/A4 (1)..(25)
CVRGIITSKTKSLDEGYNKALNELC

SEQ ID NO: 9 - protein, 25 aa, Clostridium Botulinum
  Loop BoNT/A5 (1)..(25)
CVRGIITSKTKSLDEGYNKALNDLC

SEQ ID NO: 10 - protein, 25 aa, Clostridium Botulinum
  Loop BoNT/A7 (1)..(25)
WVRGIIPFKPKSLDEGSNKALNDLC

SEQ ID NO: 11 - protein, 10 aa, Clostridium Botulinum
  Loop BoNT/B1/B4bv/B6 (1)..(10)
CKSVKAPGIC

SEQ ID NO: 12 - protein, 10 aa, Clostridium Botulinum
  Loop BoNT/B2/B3 (1)..(10)
CKSVRAPGIC

SEQ ID NO: 13 - protein, 10 aa, Clostridium Botulinum
  Loop BoNT/B5np (1)..(10)
CKSVKVPGIC

SEQ ID NO: 14 - protein, 17 aa, Clostridium Botulinum
  Loop BoNT/C/CD (1)..(17)
CHKAIDGRSLYNKTLDC

SEQ ID NO: 15 - protein, 14 aa, Clostridium Botulinum
  Loop BoNT/D (1)..(14)
CLRLTKNSRDDSTC

SEQ ID NO: 16 - protein, 14 aa, Clostridium Botulinum
  Loop BoNT/DC (1)..(14)
CLRLTRNSRDDSTC

SEQ ID NO: 17 - protein, 15 aa, Clostridium Botulinum
  Loop BoNT/E1-E5 (1)..(15)
CKNIVSVKGIRKSIC

SEQ ID NO: 18 - protein, 15 aa, Clostridium Botulinum
  Loop BoNT/E6 (1)..(15)
CKNIVFSKGIRKSIC

SEQ ID NO: 19 - protein, 17 aa, Clostridium Botulinum
  Loop BoNT/F1/F6 (1)..(17)
CKSVIPRKGTKAPPRLC

SEQ ID NO: 20 - protein, 17 aa, Clostridium Botulinum
  Loop BoNT/F2/F3 (1)..(17)
CKSIIPRKGTKQSPSLC

SEQ ID NO: 21 - protein, 17 aa, Clostridium Botulinum
  Loop BoNT/F4 (1)..(17)
CKSIIPRKGTKAPPRLC

SEQ ID NO: 22 - protein, 15 aa, Clostridium Botulinum
  Loop BoNT/F5 (1)..(15)
CLNSSFKKNTKKPLC

SEQ ID NO: 23 - protein, 15 aa, Clostridium Botulinum
  Loop BoNT/F7 (1)..(15)
CKSIVSKKGTKNSLC

SEQ ID NO: 24 - protein, 15 aa, Clostridium Botulinum
  Loop BoNT/G (1)..(15)
CKPVMYKNTGKSEQC

SEQ ID NO: 25 - protein, 29 aa, Clostridium Tetani
  Loop TeNT (1)..(29)
CKKIIPPTNIRENLYNRTASLTDLGGELC

SEQ ID NO: 26 - DNA, 1005 bp, C. Botulinum
atggttcaaggtcaaagcgttaaaggagtaggaaaaactagcttggatggactagtaaatattgatgtaacttatggaaatggaaaatactatttaaaagatagcaacaaaaatatttatctatatgacttaaaaaatcaagttgatgaatatgatctatacaattatcttagtagacctaactataaacaaatattaatgagcaaatctgaattaatatctaattacaataataattttatagccaacaatcaggttaattctgtagatgcttatgtaaacacaaataaaacctatgattattataaaaacaaattaaatagaaacagtattgataataagggtatgaatattaatgggtttgttcatgtaggtagaaattatggtaatgctttttggtacggtccatatgatgggatgttctttggcgatggcgacggaatatacttctcttcccttgcaaaatctttagatgttgtaggccacgaattaagtcatggtgtaacaaataaagagtctaatcttaaatatgaaaatgaatctggtgccctaaatgaatctttctcagatattatgggagtagctgttgagggtaaaaactttgtactaggtgaagattgctgggttgctggaggagtaatgagagatatggaaaatccatccagaggaggccaaccagctcatatgaaagattataaatacaaaactatgaatgacgataacggtggtgttcatacaaattcaggtataataaaccatgctgcttatttagttgcagatggaatagaaaaaactggtgcaaaaaatagtaaagatattatgggaaaaatattctatacagctaattgctataaatgggatgaaacaacaaattttgctaagtgcagaaatgatgtagtccaagttactaaagaactttatggcgaaaatagcaactatgtaaaaattgttgaaaaagcttttgaccaagttggaataactgctacacctcaattaccattataa

SEQ ID NO: 27 - DNA, 1746 bp, Clostridium Botulinum
atgaaaagtaaaaaattattagctacagtgctaagtgccgtgatcactttttctactgtttctgcagtttatgctgcgcctgtaggaaaagaaagtaaagttgaaccaaaaactacaacaataacttgggaaaaaaatgaacaaaatactaaaaaagctgctactgatataactgaaaagaaatttaacaattctgaggagataactaaattctttgaaaaaaatatatctaaatttggtgtacaaaaaggttctcttaaaaacaccaagactgtaaaagacgaaaaaggtaaaactaactatcatatgatttatgaagtagaaggtatacctgtatactatggaagaattgtttttacaactgaaaaagactcctccatggattctataaacggtagaattgatactgtttttgaaaatgggaattggaaaaacaaaatcaaactatcaaaagaagatgctatagcaaaagctaaaaatgatattaaagatgaaaaagcaactagtaaaaagaccgatttatatctgtataattttgagggcaaaccttatgtagtttatttagtagatctaattacagacaacgggagttggacggttttcgttaatgctgaggatggttctatagtaaataaatttaataatactcctactttaattgatactaaagatcaaaaattacccaatgctaaaaaaattaaagatgaagctaaaaaagctagtaatgcaaataatgtaattgatgttcaaggtcaaagcgttaaaggagtaggaaaaactagcttggatggactagtaaatattgatgtaacttatggaaatggaaaatactatttaaaagatagcaacaaaaatatttatctatatgacttaaaaaatcaagttgatgaatatgatctatacaattatcttagtagacctaactataaacaaatattaatgagcaaatctgaattaatatctaattacaataataattttatagccaacaatcaggttaattctgtagatgcttatgtaaacacaaataaaacctatgattattataaaaacaaattaaatagaaacagtattgataataagggtatgaatattaatgggtttgttcatgtaggtagaaattatggtaatgctttttggtacggtccatatgatgggatgttctttggcgatggcgacggaatatacttctcttcccttgcaaaatctttagatgttgtaggccacgaattaagtcatggtgtaacaaataaagagtctaatcttaaatatgaaaatgaatctggtgccctaaatgaatctttctcagatattatgggagtagctgttgagggtaaaaactttgtactaggtgaagattgctgggttgctggaggagtaatgagagatatggaaaatccatccagaggaggccaaccagctcatatgaaagattataaatacaaaactatgaatgacgataacggtggtgttcatacaaattcaggtataataaaccatgctgcttatttagttgcagatggaatagaaaaaactggtgcaaaaaatagtaaagatattatgggaaaaatattctatacagctaattgctataaatgggatgaaacaacaaattttgctaagtgcagaaatgatgtagtccaagttactaaagaactttatggcgaaaatagcaactatgtaaaaattgttgaaaaagcttttgaccaagttggaataactgctacacctcaattaccattataa